European Patent Specification EP 3 878 977 B1, published May 3, 2023. Title: DETECTING NEOPLASM. Applicant: Mayo Foundation for Medical Education and Research. The sequence listing filed with the application follows.

SEQUENCE LISTING (202 sequences)

SEQ ID NO: 1 - DNA, 21 bp, Artificial sequence
  Synthetic
gattttgttcgtcgttagtgc

SEQ ID NO: 2 - DNA, 19 bp, Artificial sequence
  Synthetic
tctctaaacccgcgaacga

SEQ ID NO: 3 - DNA, 25 bp, Artificial sequence
  Synthetic
ttcgaagtttcgggataggaagcgt

SEQ ID NO: 4 - DNA, 20 bp, Artificial sequence
  Synthetic
cctaccgaccttcgaacgcg

SEQ ID NO: 5 - DNA, 21 bp, Artificial sequence
  Synthetic
ggcggcgcgtatttttttcgc

SEQ ID NO: 6 - DNA, 23 bp, Artificial sequence
  Synthetic
cgctacgatataaacgacgacga

SEQ ID NO: 7 - DNA, 19 bp, Artificial sequence
  Synthetic
ggttcggttgtcgtagcgc

SEQ ID NO: 8 - DNA, 20 bp, Artificial sequence
  Synthetic
ccgaccgtaatcctcgacga

SEQ ID NO: 9 - DNA, 25 bp, Artificial sequence
  Synthetic
ttaggtcgggaatcgttattgtttc

SEQ ID NO: 10 - DNA, 22 bp, Artificial sequence
  Synthetic
gtaaataaccccgcgctaaacg

SEQ ID NO: 11 - DNA, 24 bp, Artificial sequence
  Synthetic
ttcgtttgtttttcgggtcgtagc

SEQ ID NO: 12 - DNA, 24 bp, Artificial sequence
  Synthetic
accacgtaacgatttactcgacga

SEQ ID NO: 13 - DNA, 23 bp, Artificial sequence
  Synthetic
cgttttcggatttgaagtcgttc

SEQ ID NO: 14 - DNA, 19 bp, Artificial sequence
  Synthetic
cgcctcgtcttccaacgaa

SEQ ID NO: 15 - DNA, 19 bp, Artificial sequence
  Synthetic
agggcgttcggttttagtc

SEQ ID NO: 16 - DNA, 22 bp, Artificial sequence
  Synthetic
aaccgaaaacgacaaaatcgat

SEQ ID NO: 17 - DNA, 21 bp, Artificial sequence
  Synthetic
tttgagcggcggtcgttgatc

SEQ ID NO: 18 - DNA, 22 bp, Artificial sequence
  Synthetic
tccccgaatctaaacgctacga

SEQ ID NO: 19 - DNA, 25 bp, Artificial sequence
  Synthetic
tttagggaagtaaagcgtcgttttc

SEQ ID NO: 20 - DNA, 22 bp, Artificial sequence
  Synthetic
aacgacgtctcgatacctacga

SEQ ID NO: 21 - DNA, 22 bp, Artificial sequence
  Synthetic
ggagagtatttcggtttttcgc

SEQ ID NO: 22 - DNA, 24 bp, Artificial sequence
  Synthetic
acaaacaaaatcgaaaaacacccg

SEQ ID NO: 23 - DNA, 23 bp, Artificial sequence
  Synthetic
gttttcgtttcggtcgaggttac

SEQ ID NO: 24 - DNA, 25 bp, Artificial sequence
  Synthetic
gccattaactcgataaaaaacgcga

SEQ ID NO: 25 - DNA, 25 bp, Artificial sequence
  Synthetic
gatttaatcgtagattcgggtcgtc

SEQ ID NO: 26 - DNA, 22 bp, Artificial sequence
  Synthetic
ccgaaacgaacgaactcaaacg

SEQ ID NO: 27 - DNA, 17 bp, Artificial sequence
  Synthetic
gcgcgtagcggcgtttc

SEQ ID NO: 28 - DNA, 19 bp, Artificial sequence
  Synthetic
cccatatcgcccgacgtaa

SEQ ID NO: 29 - DNA, 22 bp, Artificial sequence
  Synthetic
tcgtatttggcgttcggtagtc

SEQ ID NO: 30 - DNA, 21 bp, Artificial sequence
  Synthetic
cgaaatccaacgccgaaacga

SEQ ID NO: 31 - DNA, 24 bp, Artificial sequence
  Synthetic
ttgtcgttcgtcgaattcgatttc

SEQ ID NO: 32 - DNA, 23 bp, Artificial sequence
  Synthetic
aacccgacgctaaaaaacgacga

SEQ ID NO: 33 - DNA, 25 bp, Artificial sequence
  Synthetic
ttgcgttggttacgtttttttacgc

SEQ ID NO: 34 - DNA, 23 bp, Artificial sequence
  Synthetic
acgccgtacgaataacgaaacga

SEQ ID NO: 35 - DNA, 21 bp, Artificial sequence
  Synthetic
cgtttttcgggtcgggttcgc

SEQ ID NO: 36 - DNA, 19 bp, Artificial sequence
  Synthetic
tccgacgctcgactcccga

SEQ ID NO: 37 - DNA, 22 bp, Artificial sequence
  Synthetic
tcggcgtatttttcgtagacgc

SEQ ID NO: 38 - DNA, 24 bp, Artificial sequence
  Synthetic
cgcaatcttaaacgtacgcttcga

SEQ ID NO: 39 - DNA, 24 bp, Artificial sequence
  Synthetic
ggtttataaagagttcggtttcgc

SEQ ID NO: 40 - DNA, 24 bp, Artificial sequence
  Synthetic
aaaacgctaaactacccgaatacg

SEQ ID NO: 41 - DNA, 19 bp, Artificial sequence
  Synthetic
tgggcgggtttcgtcgtac

SEQ ID NO: 42 - DNA, 21 bp, Artificial sequence
  Synthetic
gtcccgaaacatcgcaaacga

SEQ ID NO: 43 - DNA, 19 bp, Artificial sequence
  Synthetic
gcgtttggattttgcgttc

SEQ ID NO: 44 - DNA, 20 bp, Artificial sequence
  Synthetic
aaaatacgccgctaccgata

SEQ ID NO: 45 - DNA, 20 bp, Artificial sequence
  Synthetic
gtttagggagtcgcggttac

SEQ ID NO: 46 - DNA, 23 bp, Artificial sequence
  Synthetic
caaatcctacgaacgaacgaacg

SEQ ID NO: 47 - DNA, 22 bp, Artificial sequence
  Synthetic
agtttggcgtagtcggtagatc

SEQ ID NO: 48 - DNA, 22 bp, Artificial sequence
  Synthetic
gcgcgcaaataccgaataaacg

SEQ ID NO: 49 - DNA, 22 bp, Artificial sequence
  Synthetic
tcggtttttagcgttcgttcgc

SEQ ID NO: 50 - DNA, 23 bp, Artificial sequence
  Synthetic
aaacaacgaaacgccaatcccga

SEQ ID NO: 51 - DNA, 25 bp, Artificial sequence
  Synthetic
tagtttttgggcgttattttcggtc

SEQ ID NO: 52 - DNA, 21 bp, Artificial sequence
  Synthetic
gcaactccgtacactcgacga

SEQ ID NO: 53 - DNA, 26 bp, Artificial sequence
  Synthetic
tttttcgtttgtttttcggtattcgc

SEQ ID NO: 54 - DNA, 22 bp, Artificial sequence
  Synthetic
cgaatcctaacgaactatccga

SEQ ID NO: 55 - DNA, 25 bp, Artificial sequence
  Synthetic
ttcggtggattttcgtattgatttc

SEQ ID NO: 56 - DNA, 24 bp, Artificial sequence
  Synthetic
aaacgaaaccgcgaactaaaacga

SEQ ID NO: 57 - DNA, 22 bp, Artificial sequence
  Synthetic
ttacgtgatagttcggggtttc

SEQ ID NO: 58 - DNA, 21 bp, Artificial sequence
  Synthetic
ataaaacgacgcgacgaaacg

SEQ ID NO: 59 - DNA, 24 bp, Artificial sequence
  Synthetic
tttcgggttttgcgttttattcgc

SEQ ID NO: 60 - DNA, 28 bp, Artificial sequence
  Synthetic
gaaaaaaaaaaacgctaaaaatacgacg

SEQ ID NO: 61 - DNA, 21 bp, Artificial sequence
  Synthetic
tagcgcgtagtggtcgtagtc

SEQ ID NO: 62 - DNA, 18 bp, Artificial sequence
  Synthetic
cctccgccgctacaaccg

SEQ ID NO: 63 - DNA, 22 bp, Artificial sequence
  Synthetic
tcgttgttttaggatcgcgttc

SEQ ID NO: 64 - DNA, 22 bp, Artificial sequence
  Synthetic
gacgaacgataaacgacgacga

SEQ ID NO: 65 - DNA, 21 bp, Artificial sequence
  Synthetic
ttcggtcgcgttgttcgttac

SEQ ID NO: 66 - DNA, 25 bp, Artificial sequence
  Synthetic
aaacgaaaaacaactcgaataacga

SEQ ID NO: 67 - DNA, 18 bp, Artificial sequence
  Synthetic
agtcggggtcggagtcgc

SEQ ID NO: 68 - DNA, 23 bp, Artificial sequence
  Synthetic
ataaatccctccgaaacccacga

SEQ ID NO: 69 - DNA, 21 bp, Artificial sequence
  Synthetic
tcggaagtgacgtagggtagc

SEQ ID NO: 70 - DNA, 19 bp, Artificial sequence
  Synthetic
cacacgcccgctaacacga

SEQ ID NO: 71 - DNA, 21 bp, Artificial sequence
  Synthetic
gcgcgttcgggtttatattgc

SEQ ID NO: 72 - DNA, 20 bp, Artificial sequence
  Synthetic
gaccaactaccgctactcga

SEQ ID NO: 73 - DNA, 20 bp, Artificial sequence
  Synthetic
aggggagaatttcgcggttc

SEQ ID NO: 74 - DNA, 24 bp, Artificial sequence
  Synthetic
aactaaattaaacctcaaccgccg

SEQ ID NO: 75 - DNA, 20 bp, Artificial sequence
  Synthetic
ttaggaggcgaggtttgcgc

SEQ ID NO: 76 - DNA, 28 bp, Artificial sequence
  Synthetic
gacgaaaccgtaacgaaaataaaaacga

SEQ ID NO: 77 - DNA, 24 bp, Artificial sequence
  Synthetic
cgaactatccgaaaaaacgacgaa

SEQ ID NO: 78 - DNA, 22 bp, Artificial sequence
  Synthetic
gcgacgcgagcgttaatttttc

SEQ ID NO: 79 - DNA, 23 bp, Artificial sequence
  Synthetic
ttcgcgtatatattcgtcgagtc

SEQ ID NO: 80 - DNA, 20 bp, Artificial sequence
  Synthetic
cacgaccactatcacgacga

SEQ ID NO: 81 - DNA, 22 bp, Artificial sequence
  Synthetic
gtacgtcggtttagttcgtagc

SEQ ID NO: 82 - DNA, 21 bp, Artificial sequence
  Synthetic
ccgaaacgcgatatcaaccga

SEQ ID NO: 83 - DNA, 20 bp, Artificial sequence
  Synthetic
cgggcggttagagggttgtc

SEQ ID NO: 84 - DNA, 26 bp, Artificial sequence
  Synthetic
ctcgaaaattcgtaaaaaccctccga

SEQ ID NO: 85 - DNA, 29 bp, Artificial sequence
  Synthetic
cgagtagtttttttttttatcgtttagac

SEQ ID NO: 86 - DNA, 24 bp, Artificial sequence
  Synthetic
caaaaaacgacacgtaaacgatcg

SEQ ID NO: 87 - DNA, 24 bp, Artificial sequence
  Synthetic
gtttcgttttgcgtttttttgcgc

SEQ ID NO: 88 - DNA, 19 bp, Artificial sequence
  Synthetic
tcccgaatcgctactccga

SEQ ID NO: 89 - DNA, 17 bp, Artificial sequence
  Synthetic
gcggttaggcgggttgc

SEQ ID NO: 90 - DNA, 25 bp, Artificial sequence
  Synthetic
attatatcaatcccaaaaacacgcg

SEQ ID NO: 91 - DNA, 22 bp, Artificial sequence
  Synthetic
tatttttcgaattcgagttcgc

SEQ ID NO: 92 - DNA, 22 bp, Artificial sequence
  Synthetic
tcacccgataaaaacgaaaacg

SEQ ID NO: 93 - DNA, 21 bp, Artificial sequence
  Synthetic
gcgtcgttagtagtacgaagc

SEQ ID NO: 94 - DNA, 21 bp, Artificial sequence
  Synthetic
gcacctcaacgaaaacaccga

SEQ ID NO: 95 - DNA, 23 bp, Artificial sequence
  Synthetic
tcgaggcggttaattttattcgc

SEQ ID NO: 96 - DNA, 23 bp, Artificial sequence
  Synthetic
gctctaacccaaatacgctacga

SEQ ID NO: 97 - DNA, 22 bp, Artificial sequence
  Synthetic
tcggtttcgaggtaagtttagc

SEQ ID NO: 98 - DNA, 23 bp, Artificial sequence
  Synthetic
cacttcgaaacaaaattacgcga

SEQ ID NO: 99 - DNA, 20 bp, Artificial sequence
  Synthetic
ggaagcggacgttttcgttc

SEQ ID NO: 100 - DNA, 22 bp, Artificial sequence
  Synthetic
acccaaaatccgaaaacgacga

SEQ ID NO: 101 - DNA, 19 bp, Artificial sequence
  Synthetic
aggttgcgggcgtgatttc

SEQ ID NO: 102 - DNA, 20 bp, Artificial sequence
  Synthetic
ccaaaaccacgcgaacacga

SEQ ID NO: 103 - DNA, 20 bp, Artificial sequence
  Synthetic
gttcggagtgtcgtagtcgc

SEQ ID NO: 104 - DNA, 21 bp, Artificial sequence
  Synthetic
aatctcgcctacgaaacgacg

SEQ ID NO: 105 - DNA, 22 bp, Artificial sequence
  Synthetic
gtttagggacgttttcgttttc

SEQ ID NO: 106 - DNA, 20 bp, Artificial sequence
  Synthetic
aacgaacgctcgataaccga

SEQ ID NO: 107 - DNA, 20 bp, Artificial sequence
  Synthetic
tttgggtcgggttaggtcgc

SEQ ID NO: 108 - DNA, 25 bp, Artificial sequence
  Synthetic
gaaaccaaaaaaacgctaactcgta

SEQ ID NO: 109 - DNA, 20 bp, Artificial sequence
  Synthetic
cgttgttggagtttggcgtc

SEQ ID NO: 110 - DNA, 21 bp, Artificial sequence
  Synthetic
tacccgaaccgcgataaaacg

SEQ ID NO: 111 - DNA, 25 bp, Artificial sequence
  Synthetic
ggtatagttcggtttttagtcgttc

SEQ ID NO: 112 - DNA, 24 bp, Artificial sequence
  Synthetic
tcttttcctccgaaaaccgaaacg

SEQ ID NO: 113 - DNA, 23 bp, Artificial sequence
  Synthetic
ggttacggttagtattcggattc

SEQ ID NO: 114 - DNA, 20 bp, Artificial sequence
  Synthetic
atatcaaccgcctacccgcg

SEQ ID NO: 115 - DNA, 24 bp, Artificial sequence
  Synthetic
ttttgttttaatgcggcggttggc

SEQ ID NO: 116 - DNA, 22 bp, Artificial sequence
  Synthetic
tatccgaactatccgctaccga

SEQ ID NO: 117 - DNA, 19 bp, Artificial sequence
  Synthetic
ggtcgcgtcgttttcgatc

SEQ ID NO: 118 - DNA, 17 bp, Artificial sequence
  Synthetic
gccgcaaacgccgacga

SEQ ID NO: 119 - DNA, 21 bp, Artificial sequence
  Synthetic
aatcggcggtagtacgagtac

SEQ ID NO: 120 - DNA, 26 bp, Artificial sequence
  Synthetic
aaaccaaatccgtaacgataataacg

SEQ ID NO: 121 - DNA, 26 bp, Artificial sequence
  Synthetic
gagttttgttttcgaaattatttcgc

SEQ ID NO: 122 - DNA, 18 bp, Artificial sequence
  Synthetic
cccgaattaccgacgacg

SEQ ID NO: 123 - DNA, 21 bp, Artificial sequence
  Synthetic
aggttcgggttcgacgatttc

SEQ ID NO: 124 - DNA, 21 bp, Artificial sequence
  Synthetic
aactctacaacgccgaaaccg

SEQ ID NO: 125 - DNA, 23 bp, Artificial sequence
  Synthetic
ttagttcgtttagcgatggcgtc

SEQ ID NO: 126 - DNA, 20 bp, Artificial sequence
  Synthetic
ccgaaactatcccgcaacga

SEQ ID NO: 127 - DNA, 21 bp, Artificial sequence
  Synthetic
ttcgtcgtttgggttatcggc

SEQ ID NO: 128 - DNA, 23 bp, Artificial sequence
  Synthetic
gccctaaaactaaaacaaccgcg

SEQ ID NO: 129 - DNA, 22 bp, Artificial sequence
  Synthetic
ggttgtcgttttagttcgtcgc

SEQ ID NO: 130 - DNA, 19 bp, Artificial sequence
  Synthetic
gcgaaaacgcccgaaccga

SEQ ID NO: 131 - DNA, 22 bp, Artificial sequence
  Synthetic
tcgtttgggagacgtattcgtc

SEQ ID NO: 132 - DNA, 25 bp, Artificial sequence
  Synthetic
actcgaaaaatttccgaactaacga

SEQ ID NO: 133 - DNA, 20 bp, Artificial sequence
  Synthetic
tcggcggttttcgttatcgc

SEQ ID NO: 134 - DNA, 21 bp, Artificial sequence
  Synthetic
ccacgaaactcgcaactacga

SEQ ID NO: 135 - DNA, 25 bp, Artificial sequence
  Synthetic
cgtttatttagcgtaatcgtttcgc

SEQ ID NO: 136 - DNA, 24 bp, Artificial sequence
  Synthetic
gaataacgaacgttcgactaccga

SEQ ID NO: 137 - DNA, 24 bp, Artificial sequence
  Synthetic
cggacgagattagttttcgttagc

SEQ ID NO: 138 - DNA, 24 bp, Artificial sequence
  Synthetic
tcgtcaatcactcgacgaaaacga

SEQ ID NO: 139 - DNA, 22 bp, Artificial sequence
  Synthetic
tcggttcgtaggtatacgtgtc

SEQ ID NO: 140 - DNA, 22 bp, Artificial sequence
  Synthetic
gctactaccaatacttccgcga

SEQ ID NO: 141 - DNA, 21 bp, Artificial sequence
  Synthetic
gttagacggttttagtttcgc

SEQ ID NO: 142 - DNA, 20 bp, Artificial sequence
  Synthetic
aaaaacccgacgacgattcg

SEQ ID NO: 143 - DNA, 21 bp, Artificial sequence
  Synthetic
gttagagttcgcgtagcgtac

SEQ ID NO: 144 - DNA, 25 bp, Artificial sequence
  Synthetic
gaaaaaaccaaccgaacgaaaacga

SEQ ID NO: 145 - DNA, 19 bp, Artificial sequence
  Synthetic
cggggcgtttcgatgtcgc

SEQ ID NO: 146 - DNA, 24 bp, Artificial sequence
  Synthetic
ccgaacgaccaaataaaaccaacg

SEQ ID NO: 147 - DNA, 22 bp, Artificial sequence
  Synthetic
cgttttatgttgggagcgttcg

SEQ ID NO: 148 - DNA, 20 bp, Artificial sequence
  Synthetic
gaccgaaccgcgtctaaacg

SEQ ID NO: 149 - DNA, 21 bp, Artificial sequence
  Synthetic
tacgtatcgaggttgcgtcgc

SEQ ID NO: 150 - DNA, 25 bp, Artificial sequence
  Synthetic
aaactctaaaacgaacgaaactcga

SEQ ID NO: 151 - DNA, 21 bp, Artificial sequence
  Synthetic
tcgagacgcgttttttgcgtc

SEQ ID NO: 152 - DNA, 20 bp, Artificial sequence
  Synthetic
aacgatcccgaaccgccgta

SEQ ID NO: 153 - DNA, 21 bp, Artificial sequence
  Synthetic
cgagtagtgcgtttttcggtc

SEQ ID NO: 154 - DNA, 22 bp, Artificial sequence
  Synthetic
gacaacaacgataacgacgacg

SEQ ID NO: 155 - DNA, 22 bp, Artificial sequence
  Synthetic
agcgtgcgttattcggttttgc

SEQ ID NO: 156 - DNA, 23 bp, Artificial sequence
  Synthetic
acctacgattcgtaaaccgaacg

SEQ ID NO: 157 - DNA, 23 bp, Artificial sequence
  Synthetic
agttcgcgtttttttcggtcgtc

SEQ ID NO: 158 - DNA, 21 bp, Artificial sequence
  Synthetic
aaccgacgcaccgactaacga

SEQ ID NO: 159 - DNA, 22 bp, Artificial sequence
  Synthetic
ttgcgtcgtttgcgtttttcgc

SEQ ID NO: 160 - DNA, 20 bp, Artificial sequence
  Synthetic
caactcgccaatctcgccga

SEQ ID NO: 161 - DNA, 18 bp, Artificial sequence
  Synthetic
tattgcggggaggtgttc

SEQ ID NO: 162 - DNA, 24 bp, Artificial sequence
  Synthetic
tcaaaaaataattaaccgaaccga

SEQ ID NO: 163 - DNA, 24 bp, Artificial sequence
  Synthetic
ttagttttcgaagttttcgttcgc

SEQ ID NO: 164 - DNA, 19 bp, Artificial sequence
  Synthetic
tccgaccctatcccgacga

SEQ ID NO: 165 - DNA, 27 bp, Artificial sequence
  Synthetic
gattagttaattaacgataaagttcgc

SEQ ID NO: 166 - DNA, 23 bp, Artificial sequence
  Synthetic
ccgaaaacgcataatatcctcga

SEQ ID NO: 167 - DNA, 26 bp, Artificial sequence
  Synthetic
ttggagagtttttcgaattttttcgc

SEQ ID NO: 168 - DNA, 19 bp, Artificial sequence
  Synthetic
gaaaaccaccctaacgccg

SEQ ID NO: 169 - DNA, 17 bp, Artificial sequence
  Synthetic
cgcggggttcgtaggtc

SEQ ID NO: 170 - DNA, 23 bp, Artificial sequence
  Synthetic
cgacaaacaacaacgaaatcgaa

SEQ ID NO: 171 - DNA, 22 bp, Artificial sequence
  Synthetic
agtagcggttatagtggcgttc

SEQ ID NO: 172 - DNA, 22 bp, Artificial sequence
  Synthetic
gcattcgcgacgaaaacaaacg

SEQ ID NO: 173 - DNA, 20 bp, Artificial sequence
  Synthetic
gtattgaggtcggcgttgtc

SEQ ID NO: 174 - DNA, 19 bp, Artificial sequence
  Synthetic
ccgcccgaataaaccgcga

SEQ ID NO: 175 - DNA, 20 bp, Artificial sequence
  Synthetic
cgtagttcggcgtagttcgc

SEQ ID NO: 176 - DNA, 21 bp, Artificial sequence
  Synthetic
aacccgcccgacgacaatacg

SEQ ID NO: 177 - DNA, 20 bp, Artificial sequence
  Synthetic
gtcgagcgcgttcgttgtac

SEQ ID NO: 178 - DNA, 22 bp, Artificial sequence
  Synthetic
gacccgaaaaataaatcccgaa

SEQ ID NO: 179 - DNA, 24 bp, Artificial sequence
  Synthetic
gatttttttagtttgttcgacggc

SEQ ID NO: 180 - DNA, 25 bp, Artificial sequence
  Synthetic
aaaattactaaacgcgaaatcgacg

SEQ ID NO: 181 - DNA, 26 bp, Artificial sequence
  Synthetic
taatgggatgataaatgtattcgcgg

SEQ ID NO: 182 - DNA, 26 bp, Artificial sequence
  Synthetic
accgcctaatccaactcgaactcgta

SEQ ID NO: 183 - DNA, 22 bp, Artificial sequence
  Synthetic
ggtgtttttaaagggtcgtcgt

SEQ ID NO: 184 - DNA, 19 bp, Artificial sequence
  Synthetic
gacccgactcctccacgta

SEQ ID NO: 185 - DNA, 30 bp, Artificial sequence
  Synthetic
ggaagtttatagtggtttcggcgggtaggc

SEQ ID NO: 186 - DNA, 22 bp, Artificial sequence
  Synthetic
gcgaaaaacgttcgaacccgcg

SEQ ID NO: 187 - DNA, 28 bp, Artificial sequence
  Synthetic
tgtcgtcgtcgcgttattttagttgttc

SEQ ID NO: 188 - DNA, 22 bp, Artificial sequence
  Synthetic
aaccgccgtccaaaccatcgta

SEQ ID NO: 189 - DNA, 25 bp, Artificial sequence
  Synthetic
gaagagttagggttcgggacgcgag

SEQ ID NO: 190 - DNA, 25 bp, Artificial sequence
  Synthetic
aacgaccaaataaacgccgaaccga

SEQ ID NO: 191 - DNA, 25 bp, Artificial sequence
  Synthetic
cgtaggagcgattaggtgggcgtcg

SEQ ID NO: 192 - DNA, 23 bp, Artificial sequence
  Synthetic
aaaccaaaacccgaaacgcgaaa

SEQ ID NO: 193 - DNA, 26 bp, Artificial sequence
  Synthetic
cgattcgggggatggattagcgttgt

SEQ ID NO: 194 - DNA, 30 bp, Artificial sequence
  Synthetic
cgaaatccccctaacgaaaatctccgaaaa

SEQ ID NO: 195 - DNA, 25 bp, Artificial sequence
  Synthetic
cggggtttttttagcgggggttttc

SEQ ID NO: 196 - DNA, 29 bp, Artificial sequence
  Synthetic
cgcgatccgaaaaataaattaacgctact

SEQ ID NO: 197 - DNA, 20 bp, Artificial sequence
  Synthetic
agcggttcgagttgggacgg

SEQ ID NO: 198 - DNA, 24 bp, Artificial sequence
  Synthetic
gaaaaacgcgatcgccgaaaacgc

SEQ ID NO: 199 - DNA, 28 bp, Artificial sequence
  Synthetic
gaaggttattaatttaatagtcgcggaa

SEQ ID NO: 200 - DNA, 25 bp, Artificial sequence
  Synthetic
aaaaaaaacgttcccgacgaccgcg

SEQ ID NO: 201 - DNA, 25 bp, Artificial sequence
  Synthetic
agttgttttatatatcggcgttcgg

SEQ ID NO: 202 - DNA, 23 bp, Artificial sequence
  Synthetic
gactatacacgcttaaccgcgaa